European Patent Specification EP 3 746 469 B1, published July 10, 2024. Title: ANTICOAGULANT PROTEINS AND THEIR USE FOR TREATING DISEASES ASSOCIATED WITH THE ACTIVATION OF NEUTROPHILS. Applicant: BIOXODES VALERIE PIREAUX STEPHANIE DEMOULIN EDMOND GODFROID JOEL TASSIGNON SANDRINE DEROCHETTE MICHEL GUYAUX. The sequence listing filed with the application follows.

SEQUENCE LISTING (3 sequences)

SEQ ID NO: 1 - protein, 67 aa, Ixodes ricinus
  polypeptide
ANHKGRGRPAKCKLPPDDGPCRARIPSYYFDRKTKTCKEFMYGGCEGNENNFENITTCQEECRAKKV

SEQ ID NO: 2 - protein, 67 aa, Ixodes ricinus
  polypeptide
ANHKGRGRPAKCKLPPDDGPCRARIPSYYFDRKTKTCKEFMYGGCEGNENNFEQITTCQEECRAKKV

SEQ ID NO: 3 - DNA, 201 bp, Ixodes ricinus
gccaaccacaaaggtagagggcggcctgcgaagtgtaaacttcctccggacgacggaccatgcagagcacgaattccgagttactactttgatagaaaaaccaaaacgtgcaaggagtttatgtatggcggatgcgaaggaaacgaaaacaattttgaaaacataactacgtgccaagaggaatgcagagcaaaaaaagtc